European Patent Application EP 4 481 051 A1, published December 25, 2024. Title: Modified D-Alulose-3-epimerase. Applicant: AMANO ENZYME INC. The sequence listing filed with the application follows.

SEQUENCE LISTING (19 sequences)

SEQ ID NO: 1 - protein, 293 aa, Asaia krungthepensis
MNKLGLHAFVWTAGWTPEDAAMAIRSTAELGYDLIEASTMDLKAFDVPATLRELEANRLGITMSFGLTADMDISSGDPERIRRGEAHLLDAISLARDVGATHVCGILYSAFQKYATPVTAEGVRGSIEVVRRVAEKAQASGITLGMEVVNRYESNVLNTARQAIAYVKRVEMPNVKLHLDCYHMNIEEADSAEAIREAGDLLGYFHTGDSHRGYLGSGSVDFPSIFRALESIQYQGPITFESFSSAVVGQPLEGILGIWRNLWEDSRDLAAHAKAFTDVQMKSAREALGRQKR

SEQ ID NO: 2 - DNA, 882 bp, synthetic construct
  misc_feature 1..882: note = Wild type sequence (codon optimized)
  source 1..882: mol_type = other DNA
atgaacaaactgggcctgcatgcgtttgtgtggaccgcgggctggaccccggaagatgcggcgatggcgattcgcagcaccgcggaactgggctatgatctgattgaagcgagcaccatggatctgaaagcgtttgatgtgccggcgaccctgcgcgaactggaagcgaaccgcctgggcattaccatgagctttggcctgaccgcggatatggatattagcagcggcgatccggaacgcattcgccgcggcgaagcgcatctgctggatgcgattagcctggcgcgcgatgtgggcgcgacccatgtgtgcggcattctgtatagcgcgtttcagaaatatgcgaccccggtgaccgcggaaggcgtgcgcggcagcattgaagtggtgcgccgcgtggcggaaaaagcgcaagcgagcggcattaccctgggcatggaagtggtgaaccgctatgaaagcaacgtgctgaacaccgcgcgccaagcgattgcgtatgtgaaacgcgtggaaatgccgaacgtgaaactgcatctggattgctatcatatgaacattgaagaagcggatagcgcggaagcgattcgcgaagcgggcgatctgctgggctattttcataccggcgatagccatcgcggctatctgggcagcggcagcgtggattttccgagcatttttcgcgcgctggaaagcattcagtatcaaggcccgattacctttgaaagctttagcagcgcggtggtgggtcagccgctggaaggcattctgggcatttggcgcaacctgtgggaagatagccgcgatctggcggcgcatgcgaaagcgtttaccgatgtgcagatgaaaagcgcgcgcgaagcgctgggccgtcagaaacgctaa

SEQ ID NO: 3 - protein, 293 aa, synthetic construct
  REGION 1..293: note = A56E mutation
MNKLGLHAFVWTAGWTPEDAAMAIRSTAELGYDLIEASTMDLKAFDVPATLRELEENRLGITMSFGLTADMDISSGDPERIRRGEAHLLDAISLARDVGATHVCGILYSAFQKYATPVTAEGVRGSIEVVRRVAEKAQASGITLGMEVVNRYESNVLNTARQAIAYVKRVEMPNVKLHLDCYHMNIEEADSAEAIREAGDLLGYFHTGDSHRGYLGSGSVDFPSIFRALESIQYQGPITFESFSSAVVGQPLEGILGIWRNLWEDSRDLAAHAKAFTDVQMKSAREALGRQKR

SEQ ID NO: 4 - protein, 293 aa, synthetic construct
  REGION 1..293: note = N57H mutation
MNKLGLHAFVWTAGWTPEDAAMAIRSTAELGYDLIEASTMDLKAFDVPATLRELEAHRLGITMSFGLTADMDISSGDPERIRRGEAHLLDAISLARDVGATHVCGILYSAFQKYATPVTAEGVRGSIEVVRRVAEKAQASGITLGMEVVNRYESNVLNTARQAIAYVKRVEMPNVKLHLDCYHMNIEEADSAEAIREAGDLLGYFHTGDSHRGYLGSGSVDFPSIFRALESIQYQGPITFESFSSAVVGQPLEGILGIWRNLWEDSRDLAAHAKAFTDVQMKSAREALGRQKR

SEQ ID NO: 5 - protein, 293 aa, synthetic construct
  REGION 1..293: note = R58G mutation
MNKLGLHAFVWTAGWTPEDAAMAIRSTAELGYDLIEASTMDLKAFDVPATLRELEANGLGITMSFGLTADMDISSGDPERIRRGEAHLLDAISLARDVGATHVCGILYSAFQKYATPVTAEGVRGSIEVVRRVAEKAQASGITLGMEVVNRYESNVLNTARQAIAYVKRVEMPNVKLHLDCYHMNIEEADSAEAIREAGDLLGYFHTGDSHRGYLGSGSVDFPSIFRALESIQYQGPITFESFSSAVVGQPLEGILGIWRNLWEDSRDLAAHAKAFTDVQMKSAREALGRQKR

SEQ ID NO: 6 - protein, 293 aa, synthetic construct
  REGION 1..293: note = F111W mutation
MNKLGLHAFVWTAGWTPEDAAMAIRSTAELGYDLIEASTMDLKAFDVPATLRELEANRLGITMSFGLTADMDISSGDPERIRRGEAHLLDAISLARDVGATHVCGILYSAWQKYATPVTAEGVRGSIEVVRRVAEKAQASGITLGMEVVNRYESNVLNTARQAIAYVKRVEMPNVKLHLDCYHMNIEEADSAEAIREAGDLLGYFHTGDSHRGYLGSGSVDFPSIFRALESIQYQGPITFESFSSAVVGQPLEGILGIWRNLWEDSRDLAAHAKAFTDVQMKSAREALGRQKR

SEQ ID NO: 7 - protein, 293 aa, synthetic construct
  REGION 1..293: note = A56E mutation, N57H mutation, R58G mutation
MNKLGLHAFVWTAGWTPEDAAMAIRSTAELGYDLIEASTMDLKAFDVPATLRELEEHGLGITMSFGLTADMDISSGDPERIRRGEAHLLDAISLARDVGATHVCGILYSAFQKYATPVTAEGVRGSIEVVRRVAEKAQASGITLGMEVVNRYESNVLNTARQAIAYVKRVEMPNVKLHLDCYHMNIEEADSAEAIREAGDLLGYFHTGDSHRGYLGSGSVDFPSIFRALESIQYQGPITFESFSSAVVGQPLEGILGIWRNLWEDSRDLAAHAKAFTDVQMKSAREALGRQKR

SEQ ID NO: 8 - protein, 293 aa, synthetic construct
  REGION 1..293: note = A56E mutation, N57H mutation, R58G mutation, F111W mutation
MNKLGLHAFVWTAGWTPEDAAMAIRSTAELGYDLIEASTMDLKAFDVPATLRELEEHGLGITMSFGLTADMDISSGDPERIRRGEAHLLDAISLARDVGATHVCGILYSAWQKYATPVTAEGVRGSIEVVRRVAEKAQASGITLGMEVVNRYESNVLNTARQAIAYVKRVEMPNVKLHLDCYHMNIEEADSAEAIREAGDLLGYFHTGDSHRGYLGSGSVDFPSIFRALESIQYQGPITFESFSSAVVGQPLEGILGIWRNLWEDSRDLAAHAKAFTDVQMKSAREALGRQKR

SEQ ID NO: 9 - DNA, 882 bp, synthetic construct
  misc_feature 1..882: note = A56E mutation (codon optimized)
  source 1..882: mol_type = other DNA
atgaacaaactgggcctgcatgcgtttgtgtggaccgcgggctggaccccggaagatgcggcgatggcgattcgcagcaccgcggaactgggctatgatctgattgaagcgagcaccatggatctgaaagcgtttgatgtgccggcgaccctgcgcgaactggaagaaaaccgcctgggcattaccatgagctttggcctgaccgcggatatggatattagcagcggcgatccggaacgcattcgccgcggcgaagcgcatctgctggatgcgattagcctggcgcgcgatgtgggcgcgacccatgtgtgcggcattctgtatagcgcgtttcagaaatatgcgaccccggtgaccgcggaaggcgtgcgcggcagcattgaagtggtgcgccgcgtggcggaaaaagcgcaagcgagcggcattaccctgggcatggaagtggtgaaccgctatgaaagcaacgtgctgaacaccgcgcgccaagcgattgcgtatgtgaaacgcgtggaaatgccgaacgtgaaactgcatctggattgctatcatatgaacattgaagaagcggatagcgcggaagcgattcgcgaagcgggcgatctgctgggctattttcataccggcgatagccatcgcggctatctgggcagcggcagcgtggattttccgagcatttttcgcgcgctggaaagcattcagtatcaaggcccgattacctttgaaagctttagcagcgcggtggtgggtcagccgctggaaggcattctgggcatttggcgcaacctgtgggaagatagccgcgatctggcggcgcatgcgaaagcgtttaccgatgtgcagatgaaaagcgcgcgcgaagcgctgggccgtcagaaacgctaa

SEQ ID NO: 10 - DNA, 882 bp, synthetic construct
  misc_feature 1..882: note = N57H mutation (codon optimized)
  source 1..882: mol_type = other DNA
atgaacaaactgggcctgcatgcgtttgtgtggaccgcgggctggaccccggaagatgcggcgatggcgattcgcagcaccgcggaactgggctatgatctgattgaagcgagcaccatggatctgaaagcgtttgatgtgccggcgaccctgcgcgaactggaagcgcatcgcctgggcattaccatgagctttggcctgaccgcggatatggatattagcagcggcgatccggaacgcattcgccgcggcgaagcgcatctgctggatgcgattagcctggcgcgcgatgtgggcgcgacccatgtgtgcggcattctgtatagcgcgtttcagaaatatgcgaccccggtgaccgcggaaggcgtgcgcggcagcattgaagtggtgcgccgcgtggcggaaaaagcgcaagcgagcggcattaccctgggcatggaagtggtgaaccgctatgaaagcaacgtgctgaacaccgcgcgccaagcgattgcgtatgtgaaacgcgtggaaatgccgaacgtgaaactgcatctggattgctatcatatgaacattgaagaagcggatagcgcggaagcgattcgcgaagcgggcgatctgctgggctattttcataccggcgatagccatcgcggctatctgggcagcggcagcgtggattttccgagcatttttcgcgcgctggaaagcattcagtatcaaggcccgattacctttgaaagctttagcagcgcggtggtgggtcagccgctggaaggcattctgggcatttggcgcaacctgtgggaagatagccgcgatctggcggcgcatgcgaaagcgtttaccgatgtgcagatgaaaagcgcgcgcgaagcgctgggccgtcagaaacgctaa

SEQ ID NO: 11 - DNA, 882 bp, synthetic construct
  misc_feature 1..882: note = R58G mutation (codon optimized)
  source 1..882: mol_type = other DNA
atgaacaaactgggcctgcatgcgtttgtgtggaccgcgggctggaccccggaagatgcggcgatggcgattcgcagcaccgcggaactgggctatgatctgattgaagcgagcaccatggatctgaaagcgtttgatgtgccggcgaccctgcgcgaactggaagcgaacggcctgggcattaccatgagctttggcctgaccgcggatatggatattagcagcggcgatccggaacgcattcgccgcggcgaagcgcatctgctggatgcgattagcctggcgcgcgatgtgggcgcgacccatgtgtgcggcattctgtatagcgcgtttcagaaatatgcgaccccggtgaccgcggaaggcgtgcgcggcagcattgaagtggtgcgccgcgtggcggaaaaagcgcaagcgagcggcattaccctgggcatggaagtggtgaaccgctatgaaagcaacgtgctgaacaccgcgcgccaagcgattgcgtatgtgaaacgcgtggaaatgccgaacgtgaaactgcatctggattgctatcatatgaacattgaagaagcggatagcgcggaagcgattcgcgaagcgggcgatctgctgggctattttcataccggcgatagccatcgcggctatctgggcagcggcagcgtggattttccgagcatttttcgcgcgctggaaagcattcagtatcaaggcccgattacctttgaaagctttagcagcgcggtggtgggtcagccgctggaaggcattctgggcatttggcgcaacctgtgggaagatagccgcgatctggcggcgcatgcgaaagcgtttaccgatgtgcagatgaaaagcgcgcgcgaagcgctgggccgtcagaaacgctaa

SEQ ID NO: 12 - DNA, 882 bp, synthetic construct
  misc_feature 1..882: note = F111W mutation (codon optimized)
  source 1..882: mol_type = other DNA
atgaacaaactgggcctgcatgcgtttgtgtggaccgcgggctggaccccggaagatgcggcgatggcgattcgcagcaccgcggaactgggctatgatctgattgaagcgagcaccatggatctgaaagcgtttgatgtgccggcgaccctgcgcgaactggaagcgaaccgcctgggcattaccatgagctttggcctgaccgcggatatggatattagcagcggcgatccggaacgcattcgccgcggcgaagcgcatctgctggatgcgattagcctggcgcgcgatgtgggcgcgacccatgtgtgcggcattctgtatagcgcgtggcagaaatatgcgaccccggtgaccgcggaaggcgtgcgcggcagcattgaagtggtgcgccgcgtggcggaaaaagcgcaagcgagcggcattaccctgggcatggaagtggtgaaccgctatgaaagcaacgtgctgaacaccgcgcgccaagcgattgcgtatgtgaaacgcgtggaaatgccgaacgtgaaactgcatctggattgctatcatatgaacattgaagaagcggatagcgcggaagcgattcgcgaagcgggcgatctgctgggctattttcataccggcgatagccatcgcggctatctgggcagcggcagcgtggattttccgagcatttttcgcgcgctggaaagcattcagtatcaaggcccgattacctttgaaagctttagcagcgcggtggtgggtcagccgctggaaggcattctgggcatttggcgcaacctgtgggaagatagccgcgatctggcggcgcatgcgaaagcgtttaccgatgtgcagatgaaaagcgcgcgcgaagcgctgggccgtcagaaacgctaa

SEQ ID NO: 13 - DNA, 882 bp, synthetic construct
  misc_feature 1..882: note = A56E mutation, N57H mutation, R58G mutation (codon optimized)
  source 1..882: mol_type = other DNA
atgaacaaactgggcctgcatgcgtttgtgtggaccgcgggctggaccccggaagatgcggcgatggcgattcgcagcaccgcggaactgggctatgatctgattgaagcgagcaccatggatctgaaagcgtttgatgtgccggcgaccctgcgcgaactggaagaacatggcctgggcattaccatgagctttggcctgaccgcggatatggatattagcagcggcgatccggaacgcattcgccgcggcgaagcgcatctgctggatgcgattagcctggcgcgcgatgtgggcgcgacccatgtgtgcggcattctgtatagcgcgtttcagaaatatgcgaccccggtgaccgcggaaggcgtgcgcggcagcattgaagtggtgcgccgcgtggcggaaaaagcgcaagcgagcggcattaccctgggcatggaagtggtgaaccgctatgaaagcaacgtgctgaacaccgcgcgccaagcgattgcgtatgtgaaacgcgtggaaatgccgaacgtgaaactgcatctggattgctatcatatgaacattgaagaagcggatagcgcggaagcgattcgcgaagcgggcgatctgctgggctattttcataccggcgatagccatcgcggctatctgggcagcggcagcgtggattttccgagcatttttcgcgcgctggaaagcattcagtatcaaggcccgattacctttgaaagctttagcagcgcggtggtgggtcagccgctggaaggcattctgggcatttggcgcaacctgtgggaagatagccgcgatctggcggcgcatgcgaaagcgtttaccgatgtgcagatgaaaagcgcgcgcgaagcgctgggccgtcagaaacgctaa

SEQ ID NO: 14 - DNA, 882 bp, synthetic construct
  misc_feature 1..882: note = A56E mutation, N57H mutation, R58G mutation, F111W mutation (codon optimized)
  source 1..882: mol_type = other DNA
atgaacaaactgggcctgcatgcgtttgtgtggaccgcgggctggaccccggaagatgcggcgatggcgattcgcagcaccgcggaactgggctatgatctgattgaagcgagcaccatggatctgaaagcgtttgatgtgccggcgaccctgcgcgaactggaagaacatggcctgggcattaccatgagctttggcctgaccgcggatatggatattagcagcggcgatccggaacgcattcgccgcggcgaagcgcatctgctggatgcgattagcctggcgcgcgatgtgggcgcgacccatgtgtgcggcattctgtatagcgcgtggcagaaatatgcgaccccggtgaccgcggaaggcgtgcgcggcagcattgaagtggtgcgccgcgtggcggaaaaagcgcaagcgagcggcattaccctgggcatggaagtggtgaaccgctatgaaagcaacgtgctgaacaccgcgcgccaagcgattgcgtatgtgaaacgcgtggaaatgccgaacgtgaaactgcatctggattgctatcatatgaacattgaagaagcggatagcgcggaagcgattcgcgaagcgggcgatctgctgggctattttcataccggcgatagccatcgcggctatctgggcagcggcagcgtggattttccgagcatttttcgcgcgctggaaagcattcagtatcaaggcccgattacctttgaaagctttagcagcgcggtggtgggtcagccgctggaaggcattctgggcatttggcgcaacctgtgggaagatagccgcgatctggcggcgcatgcgaaagcgtttaccgatgtgcagatgaaaagcgcgcgcgaagcgctgggccgtcagaaacgctaa

SEQ ID NO: 15 - DNA, 882 bp, Asaia krungthepensis
  source 1..882: mol_type = genomic DNA
atgaacaagctcggactccacgcttttgtctggactgctggctggacgcctgaagacgccgccatggccatccgctcgacggctgaactcggctacgatctgatcgaggcctcgaccatggacctcaaggccttcgacgtgcccgcaacactgcgcgaactcgaagccaatcgtctcgggatcaccatgtccttcggcttgactgcagatatggatatctcctcgggcgacccggagcgtatccgtcggggagaggcgcatctgctcgatgccatttcccttgcccgagatgtcggggcgacccatgtctgcggcattctctattccgccttccagaaatacgcgacgccggtgacggcagaaggcgtgcgcggctctatcgaagtggtgcgtcgtgtcgctgaaaaggcgcaggccagtggcatcacgctgggcatggaagtggtcaatcgctacgagtccaacgtgctcaatacggcacgtcaggcgattgcctatgtgaagcgcgtcgagatgcccaatgtgaagctgcacctcgattgctatcacatgaatatcgaagaagcggattccgccgaggccattcgcgaggcgggcgatctgctgggctatttccataccggggattcgcatcgcggctatcttggatcgggttcggtcgatttcccgagcatattccgcgcgctggagagcattcagtatcaagggccgatcactttcgaatccttctcctcagcggtggtcggtcaaccgctcgaagggattctgggcatttggcgcaatctctgggaagacagccgtgatctcgcggcccatgccaaggccttcaccgatgtgcagatgaaatcggcacgcgaggcgctcggccgccagaagcgctaa

SEQ ID NO: 16 - DNA, 30 bp, synthetic construct
  misc_feature 1..30: note = Primer
  source 1..30: mol_type = other DNA
gaagaacatggcctgggcattaccatgagc

SEQ ID NO: 17 - DNA, 30 bp, synthetic construct
  misc_feature 1..30: note = Primer
  source 1..30: mol_type = other DNA
caggccatgttcttccagttcgcgcagggt

SEQ ID NO: 18 - DNA, 27 bp, synthetic construct
  misc_feature 1..27: note = Primer
  source 1..27: mol_type = other DNA
agcgcgtggcagaaatatgcgaccccg

SEQ ID NO: 19 - DNA, 27 bp, synthetic construct
  misc_feature 1..27: note = Primer
  source 1..27: mol_type = other DNA
tttctgccacgcgctatacagaatgcc